European Patent Application EP 4 252 852 A2, published October 4, 2023. Title: METHODS AND MATERIALS FOR TREATING CANCER. Applicant: MAYO FOUNDATION FOR MEDICAL EDUCATION AND RESEARCH. Application EP. The sequence listing filed with the application follows.

SEQUENCE LISTING (575 sequences)

SEQ ID NO: 1 - DNA, 15 bp, Homo sapiens
  source 1..15: mol_type = other DNA
atgagctttgatcca

SEQ ID NO: 2 - DNA, 15 bp, synthetic construct
  misc_feature 1..15: note = Description of Artificial Sequence: Synthetic oligonucleotide
  source 1..15: mol_type = other DNA
atgagctttgattca

SEQ ID NO: 3 - protein, 9 aa, Homo sapiens
NSAANLRFV

SEQ ID NO: 4 - protein, 9 aa, synthetic construct
  REGION 1..9: note = Description of Artificial Sequence: Synthetic peptide
NSATNLRFV

SEQ ID NO: 5 - protein, 8 aa, Homo sapiens
ASFIFSKG

SEQ ID NO: 6 - protein, 8 aa, synthetic construct
  REGION 1..8: note = Description of Artificial Sequence: Synthetic peptide
TSFIFSKG

SEQ ID NO: 7 - protein, 8 aa, Homo sapiens
MSFDPNLL

SEQ ID NO: 8 - protein, 8 aa, synthetic construct
  REGION 1..8: note = Description of Artificial Sequence: Synthetic peptide
MSFDSNLL

SEQ ID NO: 9 - protein, 8 aa, Homo sapiens
RSEELCPL

SEQ ID NO: 10 - protein, 8 aa, synthetic construct
  REGION 1..8: note = Description of Artificial Sequence: Synthetic peptide
RSEEFCPL

SEQ ID NO: 11 - protein, 9 aa, Homo sapiens
SSGGWAARA

SEQ ID NO: 12 - protein, 9 aa, synthetic construct
  REGION 1..9: note = Description of Artificial Sequence: Synthetic peptide
SSGGWAARV

SEQ ID NO: 13 - protein, 9 aa, Homo sapiens
SSVIDEISV

SEQ ID NO: 14 - protein, 9 aa, synthetic construct
  REGION 1..9: note = Description of Artificial Sequence: Synthetic peptide
SSVINEISV

SEQ ID NO: 15 - protein, 9 aa, Homo sapiens
VRLKCLTAL

SEQ ID NO: 16 - protein, 9 aa, synthetic construct
  REGION 1..9: note = Description of Artificial Sequence: Synthetic peptide
VRFKCLTAL

SEQ ID NO: 17 - protein, 8 aa, Homo sapiens
TLVYLTHL

SEQ ID NO: 18 - protein, 8 aa, synthetic construct
  REGION 1..8: note = Description of Artificial Sequence: Synthetic peptide
TLVYFTHL

SEQ ID NO: 19 - protein, 9 aa, Homo sapiens
VYLTHLDYV

SEQ ID NO: 20 - protein, 9 aa, synthetic construct
  REGION 1..9: note = Description of Artificial Sequence: Synthetic peptide
VYFTHLDYV

SEQ ID NO: 21 - protein, 10 aa, Homo sapiens
RETLVYLTHL

SEQ ID NO: 22 - protein, 10 aa, synthetic construct
  REGION 1..10: note = Description of Artificial Sequence: Synthetic peptide
RETLVYFTHL

SEQ ID NO: 23 - protein, 5 aa, Homo sapiens
MSFDP

SEQ ID NO: 24 - protein, 5 aa, synthetic construct
  REGION 1..5: note = Description of Artificial Sequence: Synthetic peptide
MSFDS

SEQ ID NO: 25 - protein, 21 aa, Homo sapiens
RRFLQLNKCPACFGTSWCRRF

SEQ ID NO: 26 - protein, 21 aa, Homo sapiens
NQCGKAFARPANLQCHKRTHT

SEQ ID NO: 27 - protein, 21 aa, Homo sapiens
SGRPSGHVVSSPLIELSKIGE

SEQ ID NO: 28 - protein, 21 aa, Homo sapiens
CNPELNQEEDGDREPEVEPEA

SEQ ID NO: 29 - protein, 21 aa, Homo sapiens
PGGTFLQENPRSREEKRKATT

SEQ ID NO: 30 - protein, 21 aa, Homo sapiens
PGGTFLQENPRSRESWQVWSL

SEQ ID NO: 31 - protein, 21 aa, Homo sapiens
RPFLDLAHPRHLHSTHSELLE

SEQ ID NO: 32 - protein, 21 aa, Homo sapiens
GQQLTSEQLPTKEGYFRAVRQ

SEQ ID NO: 33 - protein, 21 aa, Homo sapiens
ECKGKQYVKRTWYKKFVGVQL

SEQ ID NO: 34 - protein, 21 aa, Homo sapiens
ALMSHELGHALGMKDVPYYTK

SEQ ID NO: 35 - protein, 21 aa, Homo sapiens
PVRIFFLYLFAICNTLQGFLI

SEQ ID NO: 36 - protein, 21 aa, Homo sapiens
GVKPEGLSLNPSQFLGDRNFA

SEQ ID NO: 37 - protein, 21 aa, Homo sapiens
ILETCKNPIQEVQSRGINIHE

SEQ ID NO: 38 - protein, 21 aa, Homo sapiens
WIIEEQPNSAANLRFVLEWTW

SEQ ID NO: 39 - protein, 21 aa, Homo sapiens
HIDIDKQKDKTGDRIITIRGG

SEQ ID NO: 40 - protein, 21 aa, Homo sapiens
DEGESPGSSHRPLTEDEIADL

SEQ ID NO: 41 - protein, 21 aa, Homo sapiens
GAWNGFVEAVELSSEEGEALR

SEQ ID NO: 42 - protein, 21 aa, Homo sapiens
EIAAKTDQKSSGKLKNGLTFR

SEQ ID NO: 43 - protein, 21 aa, Homo sapiens
MAFGPTSYRPRLLLSGERGSG

SEQ ID NO: 44 - protein, 21 aa, Homo sapiens
ETNLKRRQVVRGFSELVSEFN

SEQ ID NO: 45 - protein, 21 aa, Homo sapiens
LCQHLGKRKKMPKGLRQLKPG

SEQ ID NO: 46 - protein, 21 aa, Homo sapiens
PLWQVSTPQTRGRKQASANIF

SEQ ID NO: 47 - protein, 21 aa, Homo sapiens
QDSLLPLEEAANSGMDTSIPS

SEQ ID NO: 48 - protein, 21 aa, Homo sapiens
MDTTPDLPLTPEEYQTLLDML

SEQ ID NO: 49 - protein, 21 aa, Homo sapiens
SKQTASPSSEAKSRAQIQARA

SEQ ID NO: 50 - protein, 21 aa, Homo sapiens
QGWKSLWCGMGTIRSGLEELW

SEQ ID NO: 51 - protein, 21 aa, Homo sapiens
PRSPQSPASKASFIFSKGTKK

SEQ ID NO: 52 - protein, 21 aa, Homo sapiens
ALSGRASPVTAPSSGLHAAVR

SEQ ID NO: 53 - protein, 21 aa, Homo sapiens
AINRAKGLKHVVQCVFVAIRT

SEQ ID NO: 54 - protein, 21 aa, Homo sapiens
AKGLKHVVQCVFVAIRTIGNI

SEQ ID NO: 55 - protein, 21 aa, Homo sapiens
SFGIQSSAINVVKILRVLRVL

SEQ ID NO: 56 - protein, 21 aa, Homo sapiens
AINRAKGLKHVVQCVFVAIRT

SEQ ID NO: 57 - protein, 21 aa, Homo sapiens
SFGIQSSAINVVKILRVLRVL

SEQ ID NO: 58 - protein, 21 aa, Homo sapiens
AINRAKGLKHVVQCVFVAIRT

SEQ ID NO: 59 - protein, 21 aa, Homo sapiens
SFGIQSSAINVVKILRVLRVL

SEQ ID NO: 60 - protein, 12 aa, Homo sapiens
MDGVYSEANEEN

SEQ ID NO: 61 - protein, 21 aa, Homo sapiens
ANKSFDVLGKVEAYLKLLKSE

SEQ ID NO: 62 - protein, 21 aa, Homo sapiens
ANDFFTSANKSFDVLGKVEAY

SEQ ID NO: 63 - protein, 21 aa, Homo sapiens
TSANKSFDVLGKVEAYLKLLK

SEQ ID NO: 64 - protein, 21 aa, Homo sapiens
PRDVEMNNYRRAMQKMAEDIL

SEQ ID NO: 65 - protein, 21 aa, Homo sapiens
LTVAGGQDNVMGLKYCFRKND

SEQ ID NO: 66 - protein, 21 aa, Homo sapiens
AELQCLTVAGGQDNVMGLKYC

SEQ ID NO: 67 - protein, 21 aa, Homo sapiens
MAQAVDRDTNRPLEPPSEFIV

SEQ ID NO: 68 - protein, 17 aa, Homo sapiens
MKIPNIGNVMNKFEILG

SEQ ID NO: 69 - protein, 21 aa, Homo sapiens
PLRTRVEILHRLCDYRLDADD

SEQ ID NO: 70 - protein, 19 aa, Homo sapiens
SARFGGRPGRPRAPVPACL

SEQ ID NO: 71 - protein, 12 aa, Homo sapiens
SARFGGRPGRPR

SEQ ID NO: 72 - protein, 21 aa, Homo sapiens
ENSMWQEQILENEEAILLSSK

SEQ ID NO: 73 - protein, 21 aa, Homo sapiens
CGPNMRAGVLSSGTGPPNPRP

SEQ ID NO: 74 - protein, 21 aa, Homo sapiens
YIIKDLEKLLMIAGEERALCL

SEQ ID NO: 75 - protein, 15 aa, Homo sapiens
GTQCARIVESSAPAS

SEQ ID NO: 76 - protein, 12 aa, Homo sapiens
MSFDPNLLHNNG

SEQ ID NO: 77 - protein, 15 aa, Homo sapiens
MSFDPNLLHNNGHNG

SEQ ID NO: 78 - protein, 21 aa, Homo sapiens
RKVNQKIGSCTQQDVELHVQK

SEQ ID NO: 79 - protein, 21 aa, Homo sapiens
NLSCLLKEGSEHLFDSFEPET

SEQ ID NO: 80 - protein, 21 aa, Homo sapiens
VHDFDCLCPSGYGGKTCELVL

SEQ ID NO: 81 - protein, 21 aa, Homo sapiens
PHGLHRVFPSGFGEFPAFMEA

SEQ ID NO: 82 - protein, 21 aa, Homo sapiens
NIMHYVVPYLRNHSAHNAPSY

SEQ ID NO: 83 - protein, 21 aa, Homo sapiens
WNVDTGPDYYRDMAIEYHGVE

SEQ ID NO: 84 - protein, 21 aa, Homo sapiens
SVFSTHAGCAGAHEAEGYPAE

SEQ ID NO: 85 - protein, 21 aa, Homo sapiens
TARTQKTAYQRNRMRFAQRNL

SEQ ID NO: 86 - protein, 21 aa, Homo sapiens
SETPKLTALHTLFVREHNRLA

SEQ ID NO: 87 - protein, 21 aa, Homo sapiens
FSVELNKFYNVDLFQRGFYQI

SEQ ID NO: 88 - protein, 21 aa, Homo sapiens
FSVELNKFYNVDLFQRGKTFQ

SEQ ID NO: 89 - protein, 21 aa, Homo sapiens
AGRVRFLTGPAVLDITDRLSV

SEQ ID NO: 90 - protein, 21 aa, Homo sapiens
SREFEDVLNILHSSYLEPSSV

SEQ ID NO: 91 - protein, 21 aa, Homo sapiens
PICLSACIIGSMSQVNQRIME

SEQ ID NO: 92 - protein, 21 aa, Homo sapiens
GTVHPWRSEELCPLTCPPNSH

SEQ ID NO: 93 - protein, 21 aa, Homo sapiens
QKGIPVKGKKTKKEQKTAHFL

SEQ ID NO: 94 - protein, 21 aa, Homo sapiens
PPPPPPPLLDSVPPPPVPGNL

SEQ ID NO: 95 - protein, 21 aa, Homo sapiens
SIPVHPIGYDDAQKLLEKVKM

SEQ ID NO: 96 - protein, 21 aa, Homo sapiens
SIPVHPIGYDDAQKLLEHMGG

SEQ ID NO: 97 - protein, 21 aa, Homo sapiens
AVRPTPASGAEAPGIPKPVPG

SEQ ID NO: 98 - protein, 21 aa, Homo sapiens
QQPVKAGVKKPRRPRVRNLSD

SEQ ID NO: 99 - protein, 21 aa, Homo sapiens
IHALCHCKSAVNKDIVSVYHS

SEQ ID NO: 100 - protein, 21 aa, Homo sapiens
PRVVAASASQRLLSAPAQPAA

SEQ ID NO: 101 - protein, 21 aa, Homo sapiens
GCERRGCLLPAPLAPLFSGRL

SEQ ID NO: 102 - protein, 21 aa, Homo sapiens
LSLSLSLSLSLSLSLSPSLSL

SEQ ID NO: 103 - protein, 13 aa, Homo sapiens
WMFLIFHDFQLSC

SEQ ID NO: 104 - protein, 13 aa, Homo sapiens
WKFLIFHDFQLSS

SEQ ID NO: 105 - protein, 21 aa, Homo sapiens
HVLQWTFLNFPPFSVSPYSRS

SEQ ID NO: 106 - protein, 21 aa, Homo sapiens
HVLKCVFLIFRDFQVSRHIPG

SEQ ID NO: 107 - protein, 21 aa, Homo sapiens
HVLKCVFLIFRDFQFSCYIPS

SEQ ID NO: 108 - protein, 21 aa, Homo sapiens
HVLKCVFLIFRVFQFPRHIPG

SEQ ID NO: 109 - protein, 21 aa, Homo sapiens
QKRLKPRNTKEVCKYNDSVNS

SEQ ID NO: 110 - protein, 21 aa, Homo sapiens
KPYKCSECDKCFTEKNGLRRH

SEQ ID NO: 111 - protein, 21 aa, Homo sapiens
SECDKCFTDKGSLRVHHRIHA

SEQ ID NO: 112 - protein, 21 aa, Homo sapiens
NHCICGKYEKVLDQDSQYIVH

SEQ ID NO: 113 - protein, 21 aa, Homo sapiens
RTHTREKPYECKQCGKAFSQS

SEQ ID NO: 114 - protein, 21 aa, Homo sapiens
AHSSHLHIHERTHTREKPYEC

SEQ ID NO: 115 - protein, 21 aa, Homo sapiens
PGSEPEIDRSSAIRERTDYLW

SEQ ID NO: 116 - protein, 21 aa, Homo sapiens
ADLPSERNEGRRRWTWRMWMA

SEQ ID NO: 117 - protein, 21 aa, Homo sapiens
DISHNMRLSRASVLYEQMREC

SEQ ID NO: 118 - protein, 21 aa, Homo sapiens
VEQAGHKCPVGKKRGSLRRPA

SEQ ID NO: 119 - protein, 21 aa, Homo sapiens
VRAGGLATLNCTVTSLIPVGP

SEQ ID NO: 120 - protein, 21 aa, Homo sapiens
QKEQEALKLSECSQRQTLEAI

SEQ ID NO: 121 - protein, 21 aa, Homo sapiens
SKGQESFKKQGKIPKIPKGPS

SEQ ID NO: 122 - protein, 21 aa, Homo sapiens
LCRLFHRENGDQGETRPRQKE

SEQ ID NO: 123 - protein, 21 aa, Homo sapiens
EGPWKTVAIAADRVDKIERGG

SEQ ID NO: 124 - protein, 21 aa, Homo sapiens
KLVYSILEGQPYFSVEAQTGI

SEQ ID NO: 125 - protein, 21 aa, Homo sapiens
TPVPLDVTTGVDIRILPQNYF

SEQ ID NO: 126 - protein, 21 aa, Homo sapiens
SIIVPNYTKSLLTFKVTSDLS

SEQ ID NO: 127 - protein, 21 aa, Homo sapiens
WYHLEIRSSPGPPVDIIELHC

SEQ ID NO: 128 - protein, 21 aa, Homo sapiens
IVPNYTKSLLTFKVTSDLSIV

SEQ ID NO: 129 - protein, 21 aa, Homo sapiens
FCEEASKNICASSAKEQQSEI

SEQ ID NO: 130 - protein, 19 aa, Homo sapiens
FCEEASKNICASSAKEQQV

SEQ ID NO: 131 - protein, 20 aa, Homo sapiens
FCEEASKNICASSAKEQQVG

SEQ ID NO: 132 - protein, 21 aa, Homo sapiens
DVGDLTQEAFDLISKENPSSQ

SEQ ID NO: 133 - protein, 21 aa, Homo sapiens
CFECCIKCLGGVPYASLVATI

SEQ ID NO: 134 - protein, 21 aa, Homo sapiens
SKNAKHLAKAGIANRFRMPHL

SEQ ID NO: 135 - protein, 21 aa, Homo sapiens
CFECCIKCLGGVPYASLVATI

SEQ ID NO: 136 - protein, 21 aa, Homo sapiens
SLLDDDFSLEPLVSAFHEFEE

SEQ ID NO: 137 - protein, 21 aa, Homo sapiens
DDFSLEPLVSAFHEFEELAKQ

SEQ ID NO: 138 - protein, 21 aa, Homo sapiens
FSLEPLVSAFHEFEELAKQLQ

SEQ ID NO: 139 - protein, 21 aa, Homo sapiens
NYLGFNYEIYVAPDHKYGSPQ

SEQ ID NO: 140 - protein, 21 aa, Homo sapiens
VVNAVYAMAHALHKMQRTLCP

SEQ ID NO: 141 - protein, 21 aa, Homo sapiens
ASGLPMRNGNRHAVDISKMAL

SEQ ID NO: 142 - protein, 21 aa, Homo sapiens
SAKLHYHDSWALILHAAALWL

SEQ ID NO: 143 - protein, 21 aa, Homo sapiens
APGFLHCASFGDPHVRSFHNQ

SEQ ID NO: 144 - protein, 21 aa, Homo sapiens
QLQPVPGAAPSPSKHTSATAA

SEQ ID NO: 145 - protein, 21 aa, Homo sapiens
AVSGLGGCPYAKGASGNVATE

SEQ ID NO: 146 - protein, 15 aa, Homo sapiens
YLLQNSVKQYSGKFF

SEQ ID NO: 147 - protein, 21 aa, Homo sapiens
LPKGDFFPPERPQQLPHGLGG

SEQ ID NO: 148 - protein, 21 aa, Homo sapiens
LPKGDFFPPERPQQLPHGLGG

SEQ ID NO: 149 - protein, 21 aa, Homo sapiens
PGGGGCAGGGGGGGAGPGPSP

SEQ ID NO: 150 - protein, 21 aa, Homo sapiens
SSTSNDVSSSDFEEGPSRKRP

SEQ ID NO: 151 - protein, 21 aa, Homo sapiens
AILGKGDLIGANLSIKDQVIK

SEQ ID NO: 152 - protein, 21 aa, Homo sapiens
VIICASLKLLHLLGLIDFSED

SEQ ID NO: 153 - protein, 21 aa, Homo sapiens
YLLRLLTGSLHTDSVEDELEM

SEQ ID NO: 154 - protein, 21 aa, Homo sapiens
NDFLIEDMIPTLKAAIRAVRI

SEQ ID NO: 155 - protein, 21 aa, Homo sapiens
PPPPPPPPPPPPPPPPPPLPG

SEQ ID NO: 156 - protein, 21 aa, Homo sapiens
NQRETTMKDLDIITIPSHNVV

SEQ ID NO: 157 - protein, 21 aa, Homo sapiens
QTFCFDHAFDDKASNELVYQF

SEQ ID NO: 158 - protein, 21 aa, Homo sapiens
VNISPLEENVSESLNSLRFAS

SEQ ID NO: 159 - protein, 21 aa, Homo sapiens
TEREVWEAWAANPGNCPPAGL

SEQ ID NO: 160 - protein, 21 aa, Homo sapiens
EVMNSKLGLDVEITTYRRLLE

SEQ ID NO: 161 - protein, 21 aa, Homo sapiens
RLEPGELIPNGPFSFYGDYQS

SEQ ID NO: 162 - protein, 21 aa, Homo sapiens
EHFVTYCRYGSRISPQAEKFY

SEQ ID NO: 163 - protein, 21 aa, Homo sapiens
LETKLICIGRSDEDKYLEDFF

SEQ ID NO: 164 - protein, 21 aa, Homo sapiens
WMKNSLKVHSDSVLEQVWDIF

SEQ ID NO: 165 - protein, 15 aa, Homo sapiens
WMKNSLKVHSDSVLE

SEQ ID NO: 166 - protein, 21 aa, Homo sapiens
NTMFPPTANMLLPTGEGQSGR

SEQ ID NO: 167 - protein, 21 aa, Homo sapiens
IVLSMVESGLSEEEAQRKIWM

SEQ ID NO: 168 - protein, 21 aa, Homo sapiens
VLIPDINFNDAFENFALDFSR

SEQ ID NO: 169 - protein, 21 aa, Homo sapiens
DEDWRSQRKHVFVLSEAGKPI

SEQ ID NO: 170 - protein, 21 aa, Homo sapiens
IDSSGLRVFHTTDIRRYDAGV

SEQ ID NO: 171 - protein, 21 aa, Homo sapiens
ITSIQMLSTLPQSQHTESKST

SEQ ID NO: 172 - protein, 21 aa, Homo sapiens
KPGQSVKFRVVSMDKTLRPLN

SEQ ID NO: 173 - protein, 21 aa, Homo sapiens
GQSVKFRVVSMDKTLRPLNEL

SEQ ID NO: 174 - protein, 21 aa, Homo sapiens
KARDEVIKQLRKLQAQMKDYQ

SEQ ID NO: 175 - protein, 21 aa, Homo sapiens
GGSIMYNLFQRYKRNQIYTYI

SEQ ID NO: 176 - protein, 21 aa, Homo sapiens
VVSDSYDIYNACEKIWGEDLR

SEQ ID NO: 177 - protein, 21 aa, Homo sapiens
NTGTESASEEGDDSLLITVVP

SEQ ID NO: 178 - protein, 21 aa, Homo sapiens
LKKLSFSTQNVLSGAQEHSYM

SEQ ID NO: 179 - protein, 15 aa, Homo sapiens
MGKLENASWIHDSLM

SEQ ID NO: 180 - protein, 21 aa, Homo sapiens
HLVAADIRVAPATALTPPQGD

SEQ ID NO: 181 - protein, 21 aa, Homo sapiens
NIRQLAEMQNAAGVKSSCSRM

SEQ ID NO: 182 - protein, 21 aa, Homo sapiens
MSEQAREENVATFRGSEYLCY

SEQ ID NO: 183 - protein, 21 aa, Homo sapiens
NIRQLAEMQNAAGVKSSCSRM

SEQ ID NO: 184 - protein, 21 aa, Homo sapiens
TGYKSHAKEILHCLKNKYFKE

SEQ ID NO: 185 - protein, 21 aa, Homo sapiens
GRHKGEVSFPGGKCDPDDQDV

SEQ ID NO: 186 - protein, 21 aa, Homo sapiens
SPQVLGHILKPGTTESGALSL

SEQ ID NO: 187 - protein, 21 aa, Homo sapiens
DHEGQPRPRVPRKRGHISPKS

SEQ ID NO: 188 - protein, 21 aa, Homo sapiens
TLFFIYVRPSAISSLDLNKVV

SEQ ID NO: 189 - protein, 21 aa, Homo sapiens
SSKMSRVVCIRLISVPYVYGF

SEQ ID NO: 190 - protein, 21 aa, Homo sapiens
SYGVILFSLRSHSSEGRSKAL

SEQ ID NO: 191 - protein, 21 aa, Homo sapiens
LQLCLFFIFLAFYLITIVGNL

SEQ ID NO: 192 - protein, 21 aa, Homo sapiens
TYTVLTPFLSPIIFSLRNKEL

SEQ ID NO: 193 - protein, 21 aa, Homo sapiens
SIIVVTVFIIALSYVYILVSI

SEQ ID NO: 194 - protein, 21 aa, Homo sapiens
IYILITILKMRSTEGRHKAFS

SEQ ID NO: 195 - protein, 21 aa, Homo sapiens
TFLRGVLLIIPFIFLSKCLPY

SEQ ID NO: 196 - protein, 21 aa, Homo sapiens
ATSWILASLSALGYSMYTMQY

SEQ ID NO: 197 - protein, 21 aa, Homo sapiens
LATMSYDRYIAICKPLHYASI

SEQ ID NO: 198 - protein, 21 aa, Homo sapiens
GSHSLCPQTGSPSMVTAITIM

SEQ ID NO: 199 - protein, 12 aa, Homo sapiens
MTLGIFANCIFC

SEQ ID NO: 200 - protein, 21 aa, Homo sapiens
KNYYSLVLDSALDRETTADYK

SEQ ID NO: 201 - protein, 21 aa, Homo sapiens
QPEEEAENTKTPWLYDQEGGV

SEQ ID NO: 202 - protein, 21 aa, Homo sapiens
DYSEVTGSMGGIPEEELDSMA

SEQ ID NO: 203 - protein, 21 aa, Homo sapiens
QGLMRFNLPARICRDIELFHF

SEQ ID NO: 204 - protein, 21 aa, Homo sapiens
KQWCKPHYQNSGGGNGVDLSV

SEQ ID NO: 205 - protein, 21 aa, Homo sapiens
ILSFENNGDYMDMKQADTTQY

SEQ ID NO: 206 - protein, 21 aa, Homo sapiens
YANGIRVMSMTHTGEPGFMLY

SEQ ID NO: 207 - protein, 21 aa, Homo sapiens
EENTVPPEHSPPEMEICTVYL

SEQ ID NO: 208 - protein, 21 aa, Homo sapiens
FGSERDLERRGRSRDVEPRDR

SEQ ID NO: 209 - protein, 21 aa, Homo sapiens
SSTTTTTITTSSSRMQQPQIS

SEQ ID NO: 210 - protein, 21 aa, Homo sapiens
YVLGIGDRHSDNIMIRESGQL

SEQ ID NO: 211 - protein, 21 aa, Homo sapiens
AESPSIASTSSTEKSFPWRST

SEQ ID NO: 212 - protein, 21 aa, Homo sapiens
TYWNTRQPSNRGGCVVVRGGS

SEQ ID NO: 213 - protein, 21 aa, Homo sapiens
DGSSGGWAARALRRALALTSL

SEQ ID NO: 214 - protein, 21 aa, Homo sapiens
EKEIRSFLIEGHLINTIRVVC

SEQ ID NO: 215 - protein, 21 aa, Homo sapiens
EIVKYTKIIAMEKLYAVFTDY

SEQ ID NO: 216 - protein, 21 aa, Homo sapiens
QGQGQGLSPERVEDYGRTHRG

SEQ ID NO: 217 - protein, 21 aa, Homo sapiens
TTKTAMCTAVAGYFDIYFEKN

SEQ ID NO: 218 - protein, 21 aa, Homo sapiens
SGPAEEEDVPGSPCPDAGDPQ

SEQ ID NO: 219 - protein, 21 aa, Homo sapiens
LDQISRYYITRAKLVSKIAKY

SEQ ID NO: 220 - protein, 21 aa, Homo sapiens
LQVTRGHLDTARTRGKVSWQI

SEQ ID NO: 221 - protein, 21 aa, Homo sapiens
KKKTNNPQFDEVFYFEVTRPC

SEQ ID NO: 222 - protein, 19 aa, Homo sapiens
MKRQSERDSSPSGRGSSSS

SEQ ID NO: 223 - protein, 21 aa, Homo sapiens
LVPCHISTNLSNKQVIEVACG

SEQ ID NO: 224 - protein, 11 aa, Homo sapiens
LVPCHISTNLS

SEQ ID NO: 225 - protein, 21 aa, Homo sapiens
VIEVACGSYHSLVLTSDGEVF

SEQ ID NO: 226 - protein, 21 aa, Homo sapiens
LVPCHISTNLSNKQVIEVACG

SEQ ID NO: 227 - protein, 21 aa, Homo sapiens
IAEGVCIPRSALYMHYLDFCE

SEQ ID NO: 228 - protein, 21 aa, Homo sapiens
RREPQQVLVSSFRALWSRLWP

SEQ ID NO: 229 - protein, 21 aa, Homo sapiens
VLGHYNNFFFAAHLLDIAMGF

SEQ ID NO: 230 - protein, 21 aa, Homo sapiens
TAAAATTAAAASSSAASPHYQ

SEQ ID NO: 231 - protein, 21 aa, Homo sapiens
LVIIWNQDSVEYYTRLGALDL

SEQ ID NO: 232 - protein, 21 aa, Homo sapiens
DASKLHSSPQMAAQHNMVDDG

SEQ ID NO: 233 - skipped

SEQ ID NO: 234 - protein, 21 aa, Homo sapiens
FMNRTEFHVYLPKFQLQEDYD

SEQ ID NO: 235 - protein, 21 aa, Homo sapiens
ILKSSSVQKESCNKRNPFWKK

SEQ ID NO: 236 - protein, 21 aa, Homo sapiens
VLIILLSTMVTSITGLSTSAI

SEQ ID NO: 237 - protein, 21 aa, Homo sapiens
VIIIGLAVTVTAITGLSTSAI

SEQ ID NO: 238 - protein, 21 aa, Homo sapiens
VIIIGLSVVVTTLTGISMSAI

SEQ ID NO: 239 - protein, 21 aa, Homo sapiens
EDFFLKCRLQEQEIQRRPSVF

SEQ ID NO: 240 - protein, 21 aa, Homo sapiens
LSSLCMCVSNLHINELLPTTL

SEQ ID NO: 241 - protein, 21 aa, Homo sapiens
LLTWVNCSSVRWATRVQDIFT

SEQ ID NO: 242 - protein, 21 aa, Homo sapiens
MRGRMGSSVIDEISVEEVNKM

SEQ ID NO: 243 - protein, 21 aa, Homo sapiens
NVVRDWLGVGGPVLTPPQEHP

SEQ ID NO: 244 - protein, 21 aa, Homo sapiens
TKEEENEMYNPTFFYENLKIP

SEQ ID NO: 245 - protein, 21 aa, Homo sapiens
PFPFLMSLRDRDFISEQKFQE

SEQ ID NO: 246 - protein, 21 aa, Homo sapiens
NANFSAELLPVTCGNLKGVLH

SEQ ID NO: 247 - protein, 21 aa, Homo sapiens
FKFELQSDFAEFSESRGSTAK

SEQ ID NO: 248 - protein, 21 aa, Homo sapiens
EGRRDIGKQVEEEKPGAGKKD

SEQ ID NO: 249 - protein, 21 aa, Homo sapiens
YCAAPERRETCEHSSEAKAFH

SEQ ID NO: 250 - protein, 21 aa, Homo sapiens
TMHDKQGEVRLKCLTALQGLY

SEQ ID NO: 251 - protein, 21 aa, Homo sapiens
SLKVIGRGAFGEVRLVQKKDT

SEQ ID NO: 252 - protein, 17 aa, Homo sapiens
MKDRTQELRSAKDSDDE

SEQ ID NO: 253 - protein, 17 aa, Homo sapiens
RIQRQLEITGRTTTNEE

SEQ ID NO: 254 - protein, 21 aa, Homo sapiens
AANYLIGQKEAKRWGTAHGSI

SEQ ID NO: 255 - protein, 21 aa, Homo sapiens
VLYYEDMKKDAKGTIKKICDF

SEQ ID NO: 256 - protein, 21 aa, Homo sapiens
EESGWSSSSPTCVPIDCGLPP

SEQ ID NO: 257 - protein, 21 aa, Homo sapiens
IPQDRPTSEELLKHMFVLRER

SEQ ID NO: 258 - protein, 21 aa, Homo sapiens
TCSDMMSFLVSIASIAMLVKI

SEQ ID NO: 259 - protein, 21 aa, Homo sapiens
TESGRNSPEKGKGKIDIQAYL

SEQ ID NO: 260 - protein, 12 aa, Homo sapiens
QPDVCFLLFGSR

SEQ ID NO: 261 - protein, 21 aa, Homo sapiens
QPEKRLKAESSKTVFSCSDES

SEQ ID NO: 262 - protein, 21 aa, Homo sapiens
FTILLVVTNRDTQETLLCMAC

SEQ ID NO: 263 - protein, 21 aa, Homo sapiens
YLDCAQADSVRNLPRAFSGLT

SEQ ID NO: 264 - protein, 21 aa, Homo sapiens
NYDVLAYCIIEALANPEKERM

SEQ ID NO: 265 - protein, 21 aa, Homo sapiens
GTIDTKRNISAEEGGSVILQC

SEQ ID NO: 266 - protein, 21 aa, Homo sapiens
SLVGSSLSAFALLPLQGDRDR

SEQ ID NO: 267 - protein, 21 aa, Homo sapiens
LDRYFYHVNNDQPIDLTKGKS

SEQ ID NO: 268 - protein, 21 aa, Homo sapiens
DERDRQNARLREENARLRLEN

SEQ ID NO: 269 - protein, 21 aa, Homo sapiens
SREQFMEHLYPQRKPLVLEGL

SEQ ID NO: 270 - protein, 14 aa, Homo sapiens
METRYNLKSPAVKR

SEQ ID NO: 271 - protein, 21 aa, Homo sapiens
WGLLSHCKVRETQEYTRNVVR

SEQ ID NO: 272 - protein, 21 aa, Homo sapiens
VFGPSASHAGRLLVFPMDGSH

SEQ ID NO: 273 - protein, 21 aa, Homo sapiens
ARQAVFTAKYSEDMKHKTTLL

SEQ ID NO: 274 - protein, 21 aa, Homo sapiens
KEKILGLLSSPTGDASYQQLM

SEQ ID NO: 275 - protein, 21 aa, Homo sapiens
KRANNGKFTLRDLLVVPMQRV

SEQ ID NO: 276 - protein, 21 aa, Homo sapiens
CSTTGFSIGMRILSFAHDAVF

SEQ ID NO: 277 - protein, 21 aa, Homo sapiens
TTCILQQTTFGVAFTMALATV

SEQ ID NO: 278 - protein, 21 aa, Homo sapiens
SILASSAGMLGCIFVPKCYTI

SEQ ID NO: 279 - protein, 21 aa, Homo sapiens
CILIQVIVCAVWLRASPPSVD

SEQ ID NO: 280 - protein, 21 aa, Homo sapiens
HGQIIIVCHKGSVNAFYCVLG

SEQ ID NO: 281 - protein, 21 aa, Homo sapiens
TTSQWDVSPSMKDFTFGNEYG

SEQ ID NO: 282 - protein, 21 aa, Homo sapiens
NEYGTFAFGQHHSEISGFKHF

SEQ ID NO: 283 - protein, 21 aa, Homo sapiens
LSEPSCFWRIRNSEDSDGDLQ

SEQ ID NO: 284 - protein, 21 aa, Homo sapiens
NLNEIQDEYLGLTCAFILAAV

SEQ ID NO: 285 - protein, 21 aa, Homo sapiens
YLGLTCAFILAAVQKPIEKDY

SEQ ID NO: 286 - protein, 21 aa, Homo sapiens
PAASLQFQGLPEGVRAGPVPS

SEQ ID NO: 287 - protein, 21 aa, Homo sapiens
AACHPTKNIIASAALENDKTI

SEQ ID NO: 288 - protein, 21 aa, Homo sapiens
FENRKGLSSHARSHLRQMGVT

SEQ ID NO: 289 - protein, 21 aa, Homo sapiens
APLEWLRYFDEKELELMLCGM

SEQ ID NO: 290 - protein, 21 aa, Homo sapiens
LGITKTSKESAFKAARKYCPH

SEQ ID NO: 291 - protein, 21 aa, Homo sapiens
YKNMRETLVYLTHLDYVDTEI

SEQ ID NO: 292 - protein, 21 aa, Homo sapiens
ETSRNAGPSPAAQAPADRPVS

SEQ ID NO: 293 - protein, 21 aa, Homo sapiens
VKQKGTGKGKGRTNTISMTGG

SEQ ID NO: 294 - protein, 21 aa, Homo sapiens
QRIYHGKKPYESSKSDKCFTH

SEQ ID NO: 295 - protein, 21 aa, Homo sapiens
KIIGDASTQTDALKLPPSQPP

SEQ ID NO: 296 - protein, 21 aa, synthetic construct
  REGION 1..21: note = Description of Artificial Sequence: Synthetic peptide
RRFLQLNKCPVCFGTSWCRRF

SEQ ID NO: 297 - protein, 21 aa, synthetic construct
  REGION 1..21: note = Description of Artificial Sequence: Synthetic peptide
NQCGKAFARPTNLQCHKRTHT

SEQ ID NO: 298 - protein, 21 aa, synthetic construct
  REGION 1..21: note = Description of Artificial Sequence: Synthetic peptide
SGRPSGHVVSFPLIELSKIGE

SEQ ID NO: 299 - protein, 21 aa, synthetic construct
  REGION 1..21: note = Description of Artificial Sequence: Synthetic peptide
CNPELNQEEDEDREPEVEPEA

SEQ ID NO: 300 - protein, 21 aa, synthetic construct
  REGION 1..21: note = Description of Artificial Sequence: Synthetic peptide
PGGTFLQENPKSREEKRKATT

SEQ ID NO: 301 - protein, 21 aa, synthetic construct
  REGION 1..21: note = Description of Artificial Sequence: Synthetic peptide
PGGTFLQENPKSRESWQVWSL

SEQ ID NO: 302 - protein, 21 aa, synthetic construct
  REGION 1..21: note = Description of Artificial Sequence: Synthetic peptide
RPFLDLAHPRYLHSTHSELLE

SEQ ID NO: 303 - protein, 21 aa, synthetic construct
  REGION 1..21: note = Description of Artificial Sequence: Synthetic peptide
GQQLTSEQLPMKEGYFRAVRQ

SEQ ID NO: 304 - protein, 21 aa, synthetic construct
  REGION 1..21: note = Description of Artificial Sequence: Synthetic peptide
ECKGKQYVKRMWYKKFVGVQL

SEQ ID NO: 305 - protein, 21 aa, synthetic construct
  REGION 1..21: note = Description of Artificial Sequence: Synthetic peptide
ALMSHELGHAFGMKDVPYYTK

SEQ ID NO: 306 - protein, 21 aa, synthetic construct
  REGION 1..21: note = Description of Artificial Sequence: Synthetic peptide
PVRIFFLYLFTICNTLQGFLI

SEQ ID NO: 307 - protein, 21 aa, synthetic construct
  REGION 1..21: note = Description of Artificial Sequence: Synthetic peptide
GVKPEGLSLNSSQFLGDRNFA

SEQ ID NO: 308 - protein, 21 aa, synthetic construct
  REGION 1..21: note = Description of Artificial Sequence: Synthetic peptide
ILETCKNPIQKVQSRGINIHE

SEQ ID NO: 309 - protein, 21 aa, synthetic construct
  REGION 1..21: note = Description of Artificial Sequence: Synthetic peptide
WIIEEQPNSATNLRFVLEWTW

SEQ ID NO: 310 - protein, 21 aa, synthetic construct
  REGION 1..21: note = Description of Artificial Sequence: Synthetic peptide
HIDIDKQKDKIGDRIITIRGG

SEQ ID NO: 311 - protein, 21 aa, synthetic construct
  REGION 1..21: note = Description of Artificial Sequence: Synthetic peptide
DEGESPGSSHKPLTEDEIADL

SEQ ID NO: 312 - protein, 21 aa, synthetic construct
  REGION 1..21: note = Description of Artificial Sequence: Synthetic peptide
GAWNGFVEAVKLSSEEGEALR

SEQ ID NO: 313 - protein, 21 aa, synthetic construct
  REGION 1..21: note = Description of Artificial Sequence: Synthetic peptide
EIAAKTDQKSFGKLKNGLTFR

SEQ ID NO: 314 - protein, 21 aa, synthetic construct
  REGION 1..21: note = Description of Artificial Sequence: Synthetic peptide
MAFGPTSYRPQLLLSGERGSG

SEQ ID NO: 315 - protein, 21 aa, synthetic construct
  REGION 1..21: note = Description of Artificial Sequence: Synthetic peptide
ETNLKRRQVVCGFSELVSEFN

SEQ ID NO: 316 - protein, 21 aa, synthetic construct
  REGION 1..21: note = Description of Artificial Sequence: Synthetic peptide
LCQHLGKRKKIPKGLRQLKPG

SEQ ID NO: 317 - protein, 21 aa, synthetic construct
  REGION 1..21: note = Description of Artificial Sequence: Synthetic peptide
PLWQVSTPQTWGRKQASANIF

SEQ ID NO: 318 - protein, 21 aa, synthetic construct
  REGION 1..21: note = Description of Artificial Sequence: Synthetic peptide
QDSLLPLEEAVNSGMDTSIPS

SEQ ID NO: 319 - protein, 21 aa, synthetic construct
  REGION 1..21: note = Description of Artificial Sequence: Synthetic peptide
MDTTPDLPLTSEEYQTLLDML

SEQ ID NO: 320 - protein, 21 aa, synthetic construct
  REGION 1..21: note = Description of Artificial Sequence: Synthetic peptide
SKQTASPSSETKSRAQIQARA

SEQ ID NO: 321 - protein, 21 aa, synthetic construct
  REGION 1..21: note = Description of Artificial Sequence: Synthetic peptide
QGWKSLWCGMRTIRSGLEELW

SEQ ID NO: 322 - protein, 21 aa, synthetic construct
  REGION 1..21: note = Description of Artificial Sequence: Synthetic peptide
PRSPQSPASKTSFIFSKGTKK

SEQ ID NO: 323 - protein, 21 aa, synthetic construct
  REGION 1..21: note = Description of Artificial Sequence: Synthetic peptide
ALSGRASPVTTPSSGLHAAVR

SEQ ID NO: 324 - protein, 21 aa, synthetic construct
  REGION 1..21: note = Description of Artificial Sequence: Synthetic peptide
AINRAKGLKHIVQCVFVAIRT

SEQ ID NO: 325 - protein, 21 aa, synthetic construct
  REGION 1..21: note = Description of Artificial Sequence: Synthetic peptide
AKGLKHVVQCIFVAIRTIGNI

SEQ ID NO: 326 - protein, 21 aa, synthetic construct
  REGION 1..21: note = Description of Artificial Sequence: Synthetic peptide
SFGIQSSAINIVKILRVLRVL

SEQ ID NO: 327 - protein, 21 aa, synthetic construct
  REGION 1..21: note = Description of Artificial Sequence: Synthetic peptide
AINRAKGLKHIVQCVFVAIRT

SEQ ID NO: 328 - protein, 21 aa, synthetic construct
  REGION 1..21: note = Description of Artificial Sequence: Synthetic peptide
SFGIQSSAINIVKILRVLRVL

SEQ ID NO: 329 - protein, 21 aa, synthetic construct
  REGION 1..21: note = Description of Artificial Sequence: Synthetic peptide
AINRAKGLKHIVQCVFVAIRT

SEQ ID NO: 330 - protein, 21 aa, synthetic construct
  REGION 1..21: note = Description of Artificial Sequence: Synthetic peptide
SFGIQSSAINIVKILRVLRVL

SEQ ID NO: 331 - protein, 12 aa, synthetic construct
  REGION 1..12: note = Description of Artificial Sequence: Synthetic peptide
MNGVYSEANEEN

SEQ ID NO: 332 - protein, 21 aa, synthetic construct
  REGION 1..21: note = Description of Artificial Sequence: Synthetic peptide
ANKSFDVLGKIEAYLKLLKSE

SEQ ID NO: 333 - protein, 21 aa, synthetic construct
  REGION 1..21: note = Description of Artificial Sequence: Synthetic peptide
ANDFFTSANKLFDVLGKVEAY

SEQ ID NO: 334 - protein, 21 aa, synthetic construct
  REGION 1..21: note = Description of Artificial Sequence: Synthetic peptide
TSANKSFDVLRKVEAYLKLLK

SEQ ID NO: 335 - protein, 21 aa, synthetic construct
  REGION 1..21: note = Description of Artificial Sequence: Synthetic peptide
PRDVEMNNYRWAMQKMAEDIL

SEQ ID NO: 336 - protein, 21 aa, synthetic construct
  REGION 1..21: note = Description of Artificial Sequence: Synthetic peptide
LTVAGGQDNVIGLKYCFRKND

SEQ ID NO: 337 - protein, 21 aa, synthetic construct
  REGION 1..21: note = Description of Artificial Sequence: Synthetic peptide
AELQCLTVAGEQDNVMGLKYC

SEQ ID NO: 338 - protein, 21 aa, synthetic construct
  REGION 1..21: note = Description of Artificial Sequence: Synthetic peptide
MAQAVDRDTNKPLEPPSEFIV

SEQ ID NO: 339 - protein, 17 aa, synthetic construct
  REGION 1..17: note = Description of Artificial Sequence: Synthetic peptide
MKIPNIDNVMNKFEILG

SEQ ID NO: 340 - protein, 21 aa, synthetic construct
  REGION 1..21: note = Description of Artificial Sequence: Synthetic peptide
PLRTRVEILHHLCDYRLDADD

SEQ ID NO: 341 - protein, 19 aa, synthetic construct
  REGION 1..19: note = Description of Artificial Sequence: Synthetic peptide
SARFGGRPRRPRAPVPACL

SEQ ID NO: 342 - protein, 12 aa, synthetic construct
  REGION 1..12: note = Description of Artificial Sequence: Synthetic peptide
STRFGGRPGRPR

SEQ ID NO: 343 - protein, 21 aa, synthetic construct
  REGION 1..21: note = Description of Artificial Sequence: Synthetic peptide
ENSMWQEQILKNEEAILLSSK

SEQ ID NO: 344 - protein, 21 aa, synthetic construct
  REGION 1..21: note = Description of Artificial Sequence: Synthetic peptide
CGPNMRAGVLFSGTGPPNPRP

SEQ ID NO: 345 - protein, 21 aa, synthetic construct
  REGION 1..21: note = Description of Artificial Sequence: Synthetic peptide
YIIKDLEKLLIIAGEERALCL

SEQ ID NO: 346 - protein, 15 aa, synthetic construct
  REGION 1..15: note = Description of Artificial Sequence: Synthetic peptide
GTQCARIVESFAPAS

SEQ ID NO: 347 - protein, 12 aa, synthetic construct
  REGION 1..12: note = Description of Artificial Sequence: Synthetic peptide
MNFDPNLLHNNG

SEQ ID NO: 348 - protein, 15 aa, synthetic construct
  REGION 1..15: note = Description of Artificial Sequence: Synthetic peptide
MSFDSNLLHNNGHNG

SEQ ID NO: 349 - protein, 21 aa, synthetic construct
  REGION 1..21: note = Description of Artificial Sequence: Synthetic peptide
RKVNQKIGSCIQQDVELHVQK

SEQ ID NO: 350 - protein, 21 aa, synthetic construct
  REGION 1..21: note = Description of Artificial Sequence: Synthetic peptide
NLSCLLKEGSKHLFDSFEPET

SEQ ID NO: 351 - protein, 21 aa, synthetic construct
  REGION 1..21: note = Description of Artificial Sequence: Synthetic peptide
VHDFDCLCPSSYGGKTCELVL

SEQ ID NO: 352 - protein, 21 aa, synthetic construct
  REGION 1..21: note = Description of Artificial Sequence: Synthetic peptide
PHGLHRVFPSDFGEFPAFMEA

SEQ ID NO: 353 - protein, 21 aa, synthetic construct
  REGION 1..21: note = Description of Artificial Sequence: Synthetic peptide
NIMHYVVPYLQNHSAHNAPSY

SEQ ID NO: 354 - protein, 21 aa, synthetic construct
  REGION 1..21: note = Description of Artificial Sequence: Synthetic peptide
WNVDTGPDYYQDMAIEYHGVE

SEQ ID NO: 355 - protein, 21 aa, synthetic construct
  REGION 1..21: note = Description of Artificial Sequence: Synthetic peptide
SVFSTHAGCASAHEAEGYPAE

SEQ ID NO: 356 - protein, 21 aa, synthetic construct
  REGION 1..21: note = Description of Artificial Sequence: Synthetic peptide
TARTQKTAYQQNRMRFAQRNL

SEQ ID NO: 357 - protein, 21 aa, synthetic construct
  REGION 1..21: note = Description of Artificial Sequence: Synthetic peptide
SETPKLTALHMLFVREHNRLA

SEQ ID NO: 358 - protein, 21 aa, synthetic construct
  REGION 1..21: note = Description of Artificial Sequence: Synthetic peptide
FSVELNKFYNMDLFQRGFYQI

SEQ ID NO: 359 - protein, 21 aa, synthetic construct
  REGION 1..21: note = Description of Artificial Sequence: Synthetic peptide
FSVELNKFYNMDLFQRGKTFQ

SEQ ID NO: 360 - protein, 21 aa, synthetic construct
  REGION 1..21: note = Description of Artificial Sequence: Synthetic peptide
FSVELNKFYNMDLFQRGFYQI

SEQ ID NO: 361 - protein, 21 aa, synthetic construct
  REGION 1..21: note = Description of Artificial Sequence: Synthetic peptide
AGRVRFLTGPVVLDITDRLSV

SEQ ID NO: 362 - protein, 21 aa, synthetic construct
  REGION 1..21: note = Description of Artificial Sequence: Synthetic peptide
SREFEDVLNIFHSSYLEPSSV

SEQ ID NO: 363 - protein, 21 aa, synthetic construct
  REGION 1..21: note = Description of Artificial Sequence: Synthetic peptide
PICLSACIIGFMSQVNQRIME

SEQ ID NO: 364 - protein, 21 aa, synthetic construct
  REGION 1..21: note = Description of Artificial Sequence: Synthetic peptide
GTVHPWRSEEFCPLTCPPNSH

SEQ ID NO: 365 - protein, 21 aa, synthetic construct
  REGION 1..21: note = Description of Artificial Sequence: Synthetic peptide
QKGIPVKGKKMKKEQKTAHFL

SEQ ID NO: 366 - protein, 21 aa, synthetic construct
  REGION 1..21: note = Description of Artificial Sequence: Synthetic peptide
PPPPPPPLLDNVPPPPVPGNL

SEQ ID NO: 367 - protein, 21 aa, synthetic construct
  REGION 1..21: note = Description of Artificial Sequence: Synthetic peptide
SIPVHPIGYDNAQKLLEKVKM

SEQ ID NO: 368 - protein, 21 aa, synthetic construct
  REGION 1..21: note = Description of Artificial Sequence: Synthetic peptide
SIPVHPIGYDNAQKLLEHMGG

SEQ ID NO: 369 - protein, 21 aa, synthetic construct
  REGION 1..21: note = Description of Artificial Sequence: Synthetic peptide
AVRPTPASGAKAPGIPKPVPG

SEQ ID NO: 370 - protein, 21 aa, synthetic construct
  REGION 1..21: note = Description of Artificial Sequence: Synthetic peptide
QQPVKAGVKKLRRPRVRNLSD

SEQ ID NO: 371 - protein, 21 aa, synthetic construct
  REGION 1..21: note = Description of Artificial Sequence: Synthetic peptide
IHALCHCKSAMNKDIVSVYHS

SEQ ID NO: 372 - protein, 21 aa, synthetic construct
  REGION 1..21: note = Description of Artificial Sequence: Synthetic peptide
PRVVAASASQWLLSAPAQPAA

SEQ ID NO: 373 - protein, 21 aa, synthetic construct
  REGION 1..21: note = Description of Artificial Sequence: Synthetic peptide
GCERRGCLLPTPLAPLFSGRL

SEQ ID NO: 374 - protein, 21 aa, synthetic construct
  REGION 1..21: note = Description of Artificial Sequence: Synthetic peptide
LSLSLSLSLSFSLSLSPSLSL

SEQ ID NO: 375 - protein, 13 aa, synthetic construct
  REGION 1..13: note = Description of Artificial Sequence: Synthetic peptide
WMFLIFHDFQFSC

SEQ ID NO: 376 - protein, 13 aa, synthetic construct
  REGION 1..13: note = Description of Artificial Sequence: Synthetic peptide
WKFLIFHDFQFSS

SEQ ID NO: 377 - protein, 21 aa, synthetic construct
  REGION 1..21: note = Description of Artificial Sequence: Synthetic peptide
HVLQWTFLNFLPFSVSPYSRS

SEQ ID NO: 378 - protein, 21 aa, synthetic construct
  REGION 1..21: note = Description of Artificial Sequence: Synthetic peptide
HVLKCVFLIFCDFQVSRHIPG

SEQ ID NO: 379 - protein, 21 aa, synthetic construct
  REGION 1..21: note = Description of Artificial Sequence: Synthetic peptide
HVLKCVFLIFCDFQFSCYIPS

SEQ ID NO: 380 - protein, 21 aa, synthetic construct
  REGION 1..21: note = Description of Artificial Sequence: Synthetic peptide
HVLKCVFLIFCVFQFPRHIPG

SEQ ID NO: 381 - protein, 21 aa, synthetic construct
  REGION 1..21: note = Description of Artificial Sequence: Synthetic peptide
QKRLKPRNTKKVCKYNDSVNS

SEQ ID NO: 382 - protein, 21 aa, synthetic construct
  REGION 1..21: note = Description of Artificial Sequence: Synthetic peptide
KPYKCSECDKYFTEKNGLRRH

SEQ ID NO: 383 - protein, 21 aa, synthetic construct
  REGION 1..21: note = Description of Artificial Sequence: Synthetic peptide
SECDKCFTDKSSLRVHHRIHA

SEQ ID NO: 384 - protein, 21 aa, synthetic construct
  REGION 1..21: note = Description of Artificial Sequence: Synthetic peptide
NHCICGKYEKILDQDSQYIVH

SEQ ID NO: 385 - protein, 21 aa, synthetic construct
  REGION 1..21: note = Description of Artificial Sequence: Synthetic peptide
RTHTREKPYEYKQCGKAFSQS

SEQ ID NO: 386 - protein, 21 aa, synthetic construct
  REGION 1..21: note = Description of Artificial Sequence: Synthetic peptide
AHSSHLHIHEQTHTREKPYEC

SEQ ID NO: 387 - protein, 21 aa, synthetic construct
  REGION 1..21: note = Description of Artificial Sequence: Synthetic peptide
PGSEPEIDRSFAIRERTDYLW

SEQ ID NO: 388 - protein, 21 aa, synthetic construct
  REGION 1..21: note = Description of Artificial Sequence: Synthetic peptide
ADLPSERNEGQRRWTWRMWMA

SEQ ID NO: 389 - protein, 21 aa, synthetic construct
  REGION 1..21: note = Description of Artificial Sequence: Synthetic peptide
DISHNMRLSRTSVLYEQMREC

SEQ ID NO: 390 - protein, 21 aa, synthetic construct
  REGION 1..21: note = Description of Artificial Sequence: Synthetic peptide
VEQAGHKCPVRKKRGSLRRPA

SEQ ID NO: 391 - protein, 21 aa, synthetic construct
  REGION 1..21: note = Description of Artificial Sequence: Synthetic peptide
VRAGGLATLNYTVTSLIPVGP

SEQ ID NO: 392 - protein, 21 aa, synthetic construct
  REGION 1..21: note = Description of Artificial Sequence: Synthetic peptide
QKEQEALKLSKCSQRQTLEAI

SEQ ID NO: 393 - protein, 21 aa, synthetic construct
  REGION 1..21: note = Description of Artificial Sequence: Synthetic peptide
SKGQESFKKQEKIPKIPKGPS

SEQ ID NO: 394 - protein, 21 aa, synthetic construct
  REGION 1..21: note = Description of Artificial Sequence: Synthetic peptide
LCRLFHRENGNQGETRPRQKE

SEQ ID NO: 395 - protein, 21 aa, synthetic construct
  REGION 1..21: note = Description of Artificial Sequence: Synthetic peptide
EGPWKTVAIATDRVDKIERGG

SEQ ID NO: 396 - protein, 21 aa, synthetic construct
  REGION 1..21: note = Description of Artificial Sequence: Synthetic peptide
KLVYSILEGQSYFSVEAQTGI

SEQ ID NO: 397 - protein, 21 aa, synthetic construct
  REGION 1..21: note = Description of Artificial Sequence: Synthetic peptide
TPVPLDVTTGIDIRILPQNYF

SEQ ID NO: 398 - protein, 21 aa, synthetic construct
  REGION 1..21: note = Description of Artificial Sequence: Synthetic peptide
SIIVPNYTKSFLTFKVTSDLS

SEQ ID NO: 399 - protein, 21 aa, synthetic construct
  REGION 1..21: note = Description of Artificial Sequence: Synthetic peptide
WYHLEIRSSPRPPVDIIELHC

SEQ ID NO: 400 - protein, 21 aa, synthetic construct
  REGION 1..21: note = Description of Artificial Sequence: Synthetic peptide
IVPNYTKSLLIFKVTSDLSIV

SEQ ID NO: 401 - protein, 21 aa, synthetic construct
  REGION 1..21: note = Description of Artificial Sequence: Synthetic peptide
FCEEASKNICVSSAKEQQSEI

SEQ ID NO: 402 - protein, 19 aa, synthetic construct
  REGION 1..19: note = Description of Artificial Sequence: Synthetic peptide
FCEEASKNICVSSAKEQQV

SEQ ID NO: 403 - protein, 20 aa, synthetic construct
  REGION 1..20: note = Description of Artificial Sequence: Synthetic peptide
FCEEASKNICVSSAKEQQVG

SEQ ID NO: 404 - protein, 21 aa, synthetic construct
  REGION 1..21: note = Description of Artificial Sequence: Synthetic peptide
DVGDLTQEAFNLISKENPSSQ

SEQ ID NO: 405 - protein, 21 aa, synthetic construct
  REGION 1..21: note = Description of Artificial Sequence: Synthetic peptide
CFECCIKCLGSVPYASLVATI

SEQ ID NO: 406 - protein, 21 aa, synthetic construct
  REGION 1..21: note = Description of Artificial Sequence: Synthetic peptide
SKNAKHLAKASIANRFRMPHL

SEQ ID NO: 407 - protein, 21 aa, synthetic construct
  REGION 1..21: note = Description of Artificial Sequence: Synthetic peptide
CFECCIKCLGSVPYASLVATI

SEQ ID NO: 408 - protein, 21 aa, synthetic construct
  REGION 1..21: note = Description of Artificial Sequence: Synthetic peptide
SLLDDDFSLESLVSAFHEFEE

SEQ ID NO: 409 - protein, 21 aa, synthetic construct
  REGION 1..21: note = Description of Artificial Sequence: Synthetic peptide
DDFSLEPLVSVFHEFEELAKQ

SEQ ID NO: 410 - protein, 21 aa, synthetic construct
  REGION 1..21: note = Description of Artificial Sequence: Synthetic peptide
FSLEPLVSAFYEFEELAKQLQ

SEQ ID NO: 411 - protein, 21 aa, synthetic construct
  REGION 1..21: note = Description of Artificial Sequence: Synthetic peptide
NYLGFNYEIYIAPDHKYGSPQ

SEQ ID NO: 412 - protein, 21 aa, synthetic construct
  REGION 1..21: note = Description of Artificial Sequence: Synthetic peptide
VVNAVYAMAHVLHKMQRTLCP

SEQ ID NO: 413 - protein, 21 aa, synthetic construct
  REGION 1..21: note = Description of Artificial Sequence: Synthetic peptide
ASGLPMRNGNQHAVDISKMAL

SEQ ID NO: 414 - protein, 21 aa, synthetic construct
  REGION 1..21: note = Description of Artificial Sequence: Synthetic peptide
SAKLHYHDSWVLILHAAALWL

SEQ ID NO: 415 - protein, 21 aa, synthetic construct
  REGION 1..21: note = Description of Artificial Sequence: Synthetic peptide
APGFLHCASFEDPHVRSFHNQ

SEQ ID NO: 416 - protein, 21 aa, synthetic construct
  REGION 1..21: note = Description of Artificial Sequence: Synthetic peptide
QLQPVPGAAPNPSKHTSATAA

SEQ ID NO: 417 - protein, 21 aa, synthetic construct
  REGION 1..21: note = Description of Artificial Sequence: Synthetic peptide
AVSGLGGCPYTKGASGNVATE

SEQ ID NO: 418 - protein, 15 aa, synthetic construct
  REGION 1..15: note = Description of Artificial Sequence: Synthetic peptide
YLLQNSVKQYFGKFF

SEQ ID NO: 419 - protein, 21 aa, synthetic construct
  REGION 1..21: note = Description of Artificial Sequence: Synthetic peptide
LPKGDFFPPEHPQQLPHGLGG

SEQ ID NO: 420 - protein, 21 aa, synthetic construct
  REGION 1..21: note = Description of Artificial Sequence: Synthetic peptide
PGGGGCAGGGEGGGAGPGPSP

SEQ ID NO: 421 - protein, 21 aa, synthetic construct
  REGION 1..21: note = Description of Artificial Sequence: Synthetic peptide
SSTSNDVSSSNFEEGPSRKRP

SEQ ID NO: 422 - protein, 21 aa, synthetic construct
  REGION 1..21: note = Description of Artificial Sequence: Synthetic peptide
AILGKGDLIGTNLSIKDQVIK

SEQ ID NO: 423 - protein, 21 aa, synthetic construct
  REGION 1..21: note = Description of Artificial Sequence: Synthetic peptide
VIICASLKLLYLLGLIDFSED

SEQ ID NO: 424 - protein, 21 aa, synthetic construct
  REGION 1..21: note = Description of Artificial Sequence: Synthetic peptide
YLLRLLTGSLYTDSVEDELEM

SEQ ID NO: 425 - protein, 21 aa, synthetic construct
  REGION 1..21: note = Description of Artificial Sequence: Synthetic peptide
NDFLIEDMIPILKAAIRAVRI

SEQ ID NO: 426 - protein, 21 aa, synthetic construct
  REGION 1..21: note = Description of Artificial Sequence: Synthetic peptide
PPPPPPPPPPLPPPPPPPLPG

SEQ ID NO: 427 - protein, 21 aa, synthetic construct
  REGION 1..21: note = Description of Artificial Sequence: Synthetic peptide
NQRETTMKDLNIITIPSHNVV

SEQ ID NO: 428 - protein, 21 aa, synthetic construct
  REGION 1..21: note = Description of Artificial Sequence: Synthetic peptide
QTFCFDHAFDNKASNELVYQF

SEQ ID NO: 429 - protein, 21 aa, synthetic construct
  REGION 1..21: note = Description of Artificial Sequence: Synthetic peptide
VNISPLEENVFESLNSLRFAS

SEQ ID NO: 430 - protein, 21 aa, synthetic construct
  REGION 1..21: note = Description of Artificial Sequence: Synthetic peptide
TEREVWEAWAVNPGNCPPAGL

SEQ ID NO: 431 - protein, 21 aa, synthetic construct
  REGION 1..21: note = Description of Artificial Sequence: Synthetic peptide
EVMNSKLGLDIEITTYRRLLE

SEQ ID NO: 432 - protein, 21 aa, synthetic construct
  REGION 1..21: note = Description of Artificial Sequence: Synthetic peptide
RLEPGELIPNDPFSFYGDYQS

SEQ ID NO: 433 - protein, 21 aa, synthetic construct
  REGION 1..21: note = Description of Artificial Sequence: Synthetic peptide
EHFVTYCRYGFRISPQAEKFY

SEQ ID NO: 434 - protein, 21 aa, synthetic construct
  REGION 1..21: note = Description of Artificial Sequence: Synthetic peptide
LETKLICIGRNDEDKYLEDFF

SEQ ID NO: 435 - protein, 21 aa, synthetic construct
  REGION 1..21: note = Description of Artificial Sequence: Synthetic peptide
WMKNSLKVHSNSVLEQVWDIF

SEQ ID NO: 436 - protein, 15 aa, synthetic construct
  REGION 1..15: note = Description of Artificial Sequence: Synthetic peptide
WMKNSLKVHSNSVLE

SEQ ID NO: 437 - protein, 21 aa, synthetic construct
  REGION 1..21: note = Description of Artificial Sequence: Synthetic peptide
KFMWSEISYLTKWWDIIDIPK

SEQ ID NO: 438 - protein, 21 aa, synthetic construct
  REGION 1..21: note = Description of Artificial Sequence: Synthetic peptide
NTMFPPTANMFLPTGEGQSGR

SEQ ID NO: 439 - protein, 21 aa, synthetic construct
  REGION 1..21: note = Description of Artificial Sequence: Synthetic peptide
IVLSMVESGLLEEEAQRKIWM

SEQ ID NO: 440 - protein, 21 aa, synthetic construct
  REGION 1..21: note = Description of Artificial Sequence: Synthetic peptide
VLIPDINFNDTFENFALDFSR

SEQ ID NO: 441 - protein, 21 aa, synthetic construct
  REGION 1..21: note = Description of Artificial Sequence: Synthetic peptide
DEDWRSQRKHMFVLSEAGKPI

SEQ ID NO: 442 - protein, 21 aa, synthetic construct
  REGION 1..21: note = Description of Artificial Sequence: Synthetic peptide
IDSSGLRVFHITDIRRYDAGV

SEQ ID NO: 443 - protein, 21 aa, synthetic construct
  REGION 1..21: note = Description of Artificial Sequence: Synthetic peptide
ITSIQMLSTLSQSQHTESKST

SEQ ID NO: 444 - protein, 21 aa, synthetic construct
  REGION 1..21: note = Description of Artificial Sequence: Synthetic peptide
KPGQSVKFRVISMDKTLRPLN

SEQ ID NO: 445 - protein, 21 aa, synthetic construct
  REGION 1..21: note = Description of Artificial Sequence: Synthetic peptide
GQSVKFRVVSIDKTLRPLNEL

SEQ ID NO: 446 - protein, 21 aa, synthetic construct
  REGION 1..21: note = Description of Artificial Sequence: Synthetic peptide
KARDEVIKQLCKLQAQMKDYQ

SEQ ID NO: 447 - protein, 21 aa, synthetic construct
  REGION 1..21: note = Description of Artificial Sequence: Synthetic peptide
GGSIMYNLFQCYKRNQIYTYI

SEQ ID NO: 448 - protein, 21 aa, synthetic construct
  REGION 1..21: note = Description of Artificial Sequence: Synthetic peptide
VVSDSYDIYNVCEKIWGEDLR

SEQ ID NO: 449 - protein, 21 aa, synthetic construct
  REGION 1..21: note = Description of Artificial Sequence: Synthetic peptide
NTGTESASEEEDDSLLITVVP

SEQ ID NO: 450 - protein, 21 aa, synthetic construct
  REGION 1..21: note = Description of Artificial Sequence: Synthetic peptide
LKKLSFSTQNILSGAQEHSYM

SEQ ID NO: 451 - protein, 15 aa, synthetic construct
  REGION 1..15: note = Description of Artificial Sequence: Synthetic peptide
MGKLKNASWIHDSLM

SEQ ID NO: 452 - protein, 21 aa, synthetic construct
  REGION 1..21: note = Description of Artificial Sequence: Synthetic peptide
HLVAADIRVALATALTPPQGD

SEQ ID NO: 453 - protein, 21 aa, synthetic construct
  REGION 1..21: note = Description of Artificial Sequence: Synthetic peptide
NIRQLAEMQNTAGVKSSCSRM

SEQ ID NO: 454 - protein, 21 aa, synthetic construct
  REGION 1..21: note = Description of Artificial Sequence: Synthetic peptide
MSEQAREENVTTFRGSEYLCY

SEQ ID NO: 455 - protein, 21 aa, synthetic construct
  REGION 1..21: note = Description of Artificial Sequence: Synthetic peptide
NIRQLAEMQNTAGVKSSCSRM

SEQ ID NO: 456 - protein, 21 aa, synthetic construct
  REGION 1..21: note = Description of Artificial Sequence: Synthetic peptide
TGYKSHAKEIFHCLKNKYFKE

SEQ ID NO: 457 - protein, 21 aa, synthetic construct
  REGION 1..21: note = Description of Artificial Sequence: Synthetic peptide
GRHKGEVSFPDGKCDPDDQDV

SEQ ID NO: 458 - protein, 21 aa, synthetic construct
  REGION 1..21: note = Description of Artificial Sequence: Synthetic peptide
SPQVLGHILKSGTTESGALSL

SEQ ID NO: 459 - protein, 21 aa, synthetic construct
  REGION 1..21: note = Description of Artificial Sequence: Synthetic peptide
DHEGQPRPRVSRKRGHISPKS

SEQ ID NO: 460 - protein, 21 aa, synthetic construct
  REGION 1..21: note = Description of Artificial Sequence: Synthetic peptide
TLFFIYVRPSTISSLDLNKVV

SEQ ID NO: 461 - protein, 21 aa, synthetic construct
  REGION 1..21: note = Description of Artificial Sequence: Synthetic peptide
SSKMSRVVCICLISVPYVYGF

SEQ ID NO: 462 - protein, 21 aa, synthetic construct
  REGION 1..21: note = Description of Artificial Sequence: Synthetic peptide
SYGVILFSLRFHSSEGRSKAL

SEQ ID NO: 463 - protein, 21 aa, synthetic construct
  REGION 1..21: note = Description of Artificial Sequence: Synthetic peptide
LQLCLFFIFLVFYLITIVGNL

SEQ ID NO: 464 - protein, 21 aa, synthetic construct
  REGION 1..21: note = Description of Artificial Sequence: Synthetic peptide
TYTVLTPFLSLIIFSLRNKEL

SEQ ID NO: 465 - protein, 21 aa, synthetic construct
  REGION 1..21: note = Description of Artificial Sequence: Synthetic peptide
SIIVVTVFIIVLSYVYILVSI

SEQ ID NO: 466 - protein, 21 aa, synthetic construct
  REGION 1..21: note = Description of Artificial Sequence: Synthetic peptide
IYILITILKMHSTEGRHKAFS

SEQ ID NO: 467 - protein, 21 aa, synthetic construct
  REGION 1..21: note = Description of Artificial Sequence: Synthetic peptide
TFLRGVLLIISFIFLSKCLPY

SEQ ID NO: 468 - protein, 21 aa, synthetic construct
  REGION 1..21: note = Description of Artificial Sequence: Synthetic peptide
ATSWILASLSVLGYSMYTMQY

SEQ ID NO: 469 - protein, 21 aa, synthetic construct
  REGION 1..21: note = Description of Artificial Sequence: Synthetic peptide
LATMSYDRYIVICKPLHYASI

SEQ ID NO: 470 - protein, 21 aa, synthetic construct
  REGION 1..21: note = Description of Artificial Sequence: Synthetic peptide
GSHSLCPQTGNPSMVTAITIM

SEQ ID NO: 471 - protein, 12 aa, synthetic construct
  REGION 1..12: note = Description of Artificial Sequence: Synthetic peptide
MILGIFANCIFC

SEQ ID NO: 472 - protein, 21 aa, synthetic construct
  REGION 1..21: note = Description of Artificial Sequence: Synthetic peptide
KNYYSLVLDSTLDRETTADYK

SEQ ID NO: 473 - protein, 21 aa, synthetic construct
  REGION 1..21: note = Description of Artificial Sequence: Synthetic peptide
QPEEEAENTKIPWLYDQEGGV

SEQ ID NO: 474 - protein, 21 aa, synthetic construct
  REGION 1..21: note = Description of Artificial Sequence: Synthetic peptide
DYSEVTGSMGEIPEEELDSMA

SEQ ID NO: 475 - protein, 21 aa, synthetic construct
  REGION 1..21: note = Description of Artificial Sequence: Synthetic peptide
QGLMRFNLPAHICRDIELFHF

SEQ ID NO: 476 - protein, 21 aa, synthetic construct
  REGION 1..21: note = Description of Artificial Sequence: Synthetic peptide
KQWCKPHYQNFGGGNGVDLSV

SEQ ID NO: 477 - protein, 21 aa, synthetic construct
  REGION 1..21: note = Description of Artificial Sequence: Synthetic peptide
ILSFENNGDYIDMKQADTTQY

SEQ ID NO: 478 - protein, 21 aa, synthetic construct
  REGION 1..21: note = Description of Artificial Sequence: Synthetic peptide
YANGIRVMSMMHTGEPGFMLY

SEQ ID NO: 479 - protein, 21 aa, synthetic construct
  REGION 1..21: note = Description of Artificial Sequence: Synthetic peptide
EENTVPPEHSSPEMEICTVYL

SEQ ID NO: 480 - protein, 21 aa, synthetic construct
  REGION 1..21: note = Description of Artificial Sequence: Synthetic peptide
FGSERDLERRSRSRDVEPRDR

SEQ ID NO: 481 - protein, 21 aa, synthetic construct
  REGION 1..21: note = Description of Artificial Sequence: Synthetic peptide
SSTTTTTITTFSSRMQQPQIS

SEQ ID NO: 482 - protein, 21 aa, synthetic construct
  REGION 1..21: note = Description of Artificial Sequence: Synthetic peptide
YVLGIGDRHSNNIMIRESGQL

SEQ ID NO: 483 - protein, 21 aa, synthetic construct
  REGION 1..21: note = Description of Artificial Sequence: Synthetic peptide
AESPSIASTSLTEKSFPWRST

SEQ ID NO: 484 - protein, 21 aa, synthetic construct
  REGION 1..21: note = Description of Artificial Sequence: Synthetic peptide
TYWNTRQPSNHGGCVVVRGGS

SEQ ID NO: 485 - protein, 21 aa, synthetic construct
  REGION 1..21: note = Description of Artificial Sequence: Synthetic peptide
DGSSGGWAARVLRRALALTSL

SEQ ID NO: 486 - protein, 21 aa, synthetic construct
  REGION 1..21: note = Description of Artificial Sequence: Synthetic peptide
EKEIRSFLIESHLINTIRVVC

SEQ ID NO: 487 - protein, 21 aa, synthetic construct
  REGION 1..21: note = Description of Artificial Sequence: Synthetic peptide
EIVKYTKIIAIEKLYAVFTDY

SEQ ID NO: 488 - protein, 21 aa, synthetic construct
  REGION 1..21: note = Description of Artificial Sequence: Synthetic peptide
QGQGQGLSPEHVEDYGRTHRG

SEQ ID NO: 489 - protein, 21 aa, synthetic construct
  REGION 1..21: note = Description of Artificial Sequence: Synthetic peptide
TTKTAMCTAVVGYFDIYFEKN

SEQ ID NO: 490 - protein, 21 aa, synthetic construct
  REGION 1..21: note = Description of Artificial Sequence: Synthetic peptide
SGPAEEEDVPRSPCPDAGDPQ

SEQ ID NO: 491 - protein, 21 aa, synthetic construct
  REGION 1..21: note = Description of Artificial Sequence: Synthetic peptide
LDQISRYYITKAKLVSKIAKY

SEQ ID NO: 492 - protein, 21 aa, synthetic construct
  REGION 1..21: note = Description of Artificial Sequence: Synthetic peptide
LQVTRGHLDTTRTRGKVSWQI

SEQ ID NO: 493 - protein, 21 aa, synthetic construct
  REGION 1..21: note = Description of Artificial Sequence: Synthetic peptide
KKKTNNPQFDKVFYFEVTRPC

SEQ ID NO: 494 - protein, 19 aa, synthetic construct
  REGION 1..19: note = Description of Artificial Sequence: Synthetic peptide
MKRQSERDFSPSGRGSSSS

SEQ ID NO: 495 - protein, 21 aa, synthetic construct
  REGION 1..21: note = Description of Artificial Sequence: Synthetic peptide
LVPCHISTNLLNKQVIEVACG

SEQ ID NO: 496 - protein, 11 aa, synthetic construct
  REGION 1..11: note = Description of Artificial Sequence: Synthetic peptide
LVPCHISTNLL

SEQ ID NO: 497 - protein, 21 aa, synthetic construct
  REGION 1..21: note = Description of Artificial Sequence: Synthetic peptide
VIEVACGSYHLLVLTSDGEVF

SEQ ID NO: 498 - protein, 21 aa, synthetic construct
  REGION 1..21: note = Description of Artificial Sequence: Synthetic peptide
LVPCHISTNLLNKQVIEVACG

SEQ ID NO: 499 - protein, 21 aa, synthetic construct
  REGION 1..21: note = Description of Artificial Sequence: Synthetic peptide
IAEGVCIPRSTLYMHYLDFCE

SEQ ID NO: 500 - protein, 21 aa, synthetic construct
  REGION 1..21: note = Description of Artificial Sequence: Synthetic peptide
RREPQQVLVSFFRALWSRLWP

SEQ ID NO: 501 - protein, 21 aa, synthetic construct
  REGION 1..21: note = Description of Artificial Sequence: Synthetic peptide
VLGHYNNFFFVAHLLDIAMGF

SEQ ID NO: 502 - protein, 21 aa, synthetic construct
  REGION 1..21: note = Description of Artificial Sequence: Synthetic peptide
TAAAATTAAATSSSAASPHYQ

SEQ ID NO: 503 - protein, 21 aa, synthetic construct
  REGION 1..21: note = Description of Artificial Sequence: Synthetic peptide
LVIIWNQDSVKYYTRLGALDL

SEQ ID NO: 504 - protein, 21 aa, synthetic construct
  REGION 1..21: note = Description of Artificial Sequence: Synthetic peptide
DASKLHSSPQIAAQHNMVDDG

SEQ ID NO: 505 - protein, 21 aa, synthetic construct
  REGION 1..21: note = Description of Artificial Sequence: Synthetic peptide
FMNRTEFHVYFPKFQLQEDYD

SEQ ID NO: 506 - protein, 21 aa, synthetic construct
  REGION 1..21: note = Description of Artificial Sequence: Synthetic peptide
ILKSSSVQKEFCNKRNPFWKK

SEQ ID NO: 507 - protein, 21 aa, synthetic construct
  REGION 1..21: note = Description of Artificial Sequence: Synthetic peptide
VLIILLSTMVISITGLSTSAI

SEQ ID NO: 508 - protein, 21 aa, synthetic construct
  REGION 1..21: note = Description of Artificial Sequence: Synthetic peptide
VIIIGLAVTVIAITGLSTSAI

SEQ ID NO: 509 - protein, 21 aa, synthetic construct
  REGION 1..21: note = Description of Artificial Sequence: Synthetic peptide
VIIIGLSVVVITLTGISMSAI

SEQ ID NO: 510 - protein, 21 aa, synthetic construct
  REGION 1..21: note = Description of Artificial Sequence: Synthetic peptide
EDFFLKCRLQKQEIQRRPSVF

SEQ ID NO: 511 - protein, 21 aa, synthetic construct
  REGION 1..21: note = Description of Artificial Sequence: Synthetic peptide
LSSLCMCVSNFHINELLPTTL

SEQ ID NO: 512 - protein, 21 aa, synthetic construct
  REGION 1..21: note = Description of Artificial Sequence: Synthetic peptide
LLTWVNCSSVQWATRVQDIFT

SEQ ID NO: 513 - protein, 21 aa, synthetic construct
  REGION 1..21: note = Description of Artificial Sequence: Synthetic peptide
MRGRMGSSVINEISVEEVNKM

SEQ ID NO: 514 - protein, 21 aa, synthetic construct
  REGION 1..21: note = Description of Artificial Sequence: Synthetic peptide
NVVRDWLGVGDPVLTPPQEHP

SEQ ID NO: 515 - protein, 21 aa, synthetic construct
  REGION 1..21: note = Description of Artificial Sequence: Synthetic peptide
TKEEENEMYNSTFFYENLKIP

SEQ ID NO: 516 - protein, 21 aa, synthetic construct
  REGION 1..21: note = Description of Artificial Sequence: Synthetic peptide
PFPFLMSLRDQDFISEQKFQE

SEQ ID NO: 517 - protein, 21 aa, synthetic construct
  REGION 1..21: note = Description of Artificial Sequence: Synthetic peptide
NANFSAELLPMTCGNLKGVLH

SEQ ID NO: 518 - protein, 21 aa, synthetic construct
  REGION 1..21: note = Description of Artificial Sequence: Synthetic peptide
FKFELQSDFAKFSESRGSTAK

SEQ ID NO: 519 - protein, 21 aa, synthetic construct
  REGION 1..21: note = Description of Artificial Sequence: Synthetic peptide
EGRRDIGKQVKEEKPGAGKKD

SEQ ID NO: 520 - protein, 21 aa, synthetic construct
  REGION 1..21: note = Description of Artificial Sequence: Synthetic peptide
YCAAPERRETYEHSSEAKAFH

SEQ ID NO: 521 - protein, 21 aa, synthetic construct
  REGION 1..21: note = Description of Artificial Sequence: Synthetic peptide
TMHDKQGEVRFKCLTALQGLY

SEQ ID NO: 522 - protein, 21 aa, synthetic construct
  REGION 1..21: note = Description of Artificial Sequence: Synthetic peptide
SLKVIGRGAFSEVRLVQKKDT

SEQ ID NO: 523 - protein, 17 aa, synthetic construct
  REGION 1..17: note = Description of Artificial Sequence: Synthetic peptide
MKDRTQKLRSAKDSDDE

SEQ ID NO: 524 - protein, 17 aa, synthetic construct
  REGION 1..17: note = Description of Artificial Sequence: Synthetic peptide
RIQRQLKITGRTTTNEE

SEQ ID NO: 525 - protein, 21 aa, synthetic construct
  REGION 1..21: note = Description of Artificial Sequence: Synthetic peptide
AANYLIGQKEVKRWGTAHGSI

SEQ ID NO: 526 - protein, 21 aa, synthetic construct
  REGION 1..21: note = Description of Artificial Sequence: Synthetic peptide
VLYYEDMKKDTKGTIKKICDF

SEQ ID NO: 527 - protein, 21 aa, synthetic construct
  REGION 1..21: note = Description of Artificial Sequence: Synthetic peptide
EESGWSSSSPICVPIDCGLPP

SEQ ID NO: 528 - protein, 21 aa, synthetic construct
  REGION 1..21: note = Description of Artificial Sequence: Synthetic peptide
IPQDRPTSEEFLKHMFVLRER

SEQ ID NO: 529 - protein, 21 aa, synthetic construct
  REGION 1..21: note = Description of Artificial Sequence: Synthetic peptide
TCSDMMSFLVNIASIAMLVKI

SEQ ID NO: 530 - protein, 21 aa, synthetic construct
  REGION 1..21: note = Description of Artificial Sequence: Synthetic peptide
TESGRNSPEKDKGKIDIQAYL

SEQ ID NO: 531 - protein, 12 aa, synthetic construct
  REGION 1..12: note = Description of Artificial Sequence: Synthetic peptide
QPDVCFLLFGLR

SEQ ID NO: 532 - protein, 21 aa, synthetic construct
  REGION 1..21: note = Description of Artificial Sequence: Synthetic peptide
QPEKRLKAESLKTVFSCSDES

SEQ ID NO: 533 - protein, 21 aa, synthetic construct
  REGION 1..21: note = Description of Artificial Sequence: Synthetic peptide
FTILLVVTNRNTQETLLCMAC

SEQ ID NO: 534 - protein, 21 aa, synthetic construct
  REGION 1..21: note = Description of Artificial Sequence: Synthetic peptide
YLDCAQADSVCNLPRAFSGLT

SEQ ID NO: 535 - protein, 21 aa, synthetic construct
  REGION 1..21: note = Description of Artificial Sequence: Synthetic peptide
NYDVLAYCIIKALANPEKERM

SEQ ID NO: 536 - protein, 21 aa, synthetic construct
  REGION 1..21: note = Description of Artificial Sequence: Synthetic peptide
GTIDTKRNISVEEGGSVILQC

SEQ ID NO: 537 - protein, 21 aa, synthetic construct
  REGION 1..21: note = Description of Artificial Sequence: Synthetic peptide
SLVGSSLSAFTLLPLQGDRDR

SEQ ID NO: 538 - protein, 21 aa, synthetic construct
  REGION 1..21: note = Description of Artificial Sequence: Synthetic peptide
LDRYFYHVNNNQPIDLTKGKS

SEQ ID NO: 539 - protein, 21 aa, synthetic construct
  REGION 1..21: note = Description of Artificial Sequence: Synthetic peptide
DERDRQNARLHEENARLRLEN

SEQ ID NO: 540 - protein, 21 aa, synthetic construct
  REGION 1..21: note = Description of Artificial Sequence: Synthetic peptide
SREQFMEHLYSQRKPLVLEGL

SEQ ID NO: 541 - protein, 14 aa, synthetic construct
  REGION 1..14: note = Description of Artificial Sequence: Synthetic peptide
METCYNLKSPAVKR

SEQ ID NO: 542 - protein, 21 aa, synthetic construct
  REGION 1..21: note = Description of Artificial Sequence: Synthetic peptide
WGLLSHCKVRKTQEYTRNVVR

SEQ ID NO: 543 - protein, 21 aa, synthetic construct
  REGION 1..21: note = Description of Artificial Sequence: Synthetic peptide
VFGPSASHAGKLLVFPMDGSH

SEQ ID NO: 544 - protein, 21 aa, synthetic construct
  REGION 1..21: note = Description of Artificial Sequence: Synthetic peptide
ARQAVFTAKYLEDMKHKTTLL

SEQ ID NO: 545 - protein, 21 aa, synthetic construct
  REGION 1..21: note = Description of Artificial Sequence: Synthetic peptide
KEKILGLLSSSTGDASYQQLM

SEQ ID NO: 546 - protein, 21 aa, synthetic construct
  REGION 1..21: note = Description of Artificial Sequence: Synthetic peptide
KRANNGKFTLHDLLVVPMQRV

SEQ ID NO: 547 - protein, 21 aa, synthetic construct
  REGION 1..21: note = Description of Artificial Sequence: Synthetic peptide
CSTTGFSIGMHILSFAHDAVF

SEQ ID NO: 548 - protein, 21 aa, synthetic construct
  REGION 1..21: note = Description of Artificial Sequence: Synthetic peptide
TTCILQQTTFEVAFTMALATV

SEQ ID NO: 549 - protein, 21 aa, synthetic construct
  REGION 1..21: note = Description of Artificial Sequence: Synthetic peptide
SILASSAGMLECIFVPKCYTI

SEQ ID NO: 550 - protein, 21 aa, synthetic construct
  REGION 1..21: note = Description of Artificial Sequence: Synthetic peptide
CILIQVIVCAIWLRASPPSVD

SEQ ID NO: 551 - protein, 21 aa, synthetic construct
  REGION 1..21: note = Description of Artificial Sequence: Synthetic peptide
HGQIIIVCHKDSVNAFYCVLG

SEQ ID NO: 552 - protein, 21 aa, synthetic construct
  REGION 1..21: note = Description of Artificial Sequence: Synthetic peptide
TTSQWDVSPSIKDFTFGNEYG

SEQ ID NO: 553 - protein, 21 aa, synthetic construct
  REGION 1..21: note = Description of Artificial Sequence: Synthetic peptide
NEYGTFAFGQYHSEISGFKHF

SEQ ID NO: 554 - protein, 21 aa, synthetic construct
  REGION 1..21: note = Description of Artificial Sequence: Synthetic peptide
LSEPSCFWRIKNSEDSDGDLQ

SEQ ID NO: 555 - protein, 21 aa, synthetic construct
  REGION 1..21: note = Description of Artificial Sequence: Synthetic peptide
NLNEIQDEYLELTCAFILAAV

SEQ ID NO: 556 - protein, 21 aa, synthetic construct
  REGION 1..21: note = Description of Artificial Sequence: Synthetic peptide
YLGLTCAFILVAVQKPIEKDY

SEQ ID NO: 557 - protein, 21 aa, synthetic construct
  REGION 1..21: note = Description of Artificial Sequence: Synthetic peptide
PAASLQFQGLSEGVRAGPVPS

SEQ ID NO: 558 - protein, 21 aa, synthetic construct
  REGION 1..21: note = Description of Artificial Sequence: Synthetic peptide
AACHPTKNIITSAALENDKTI

SEQ ID NO: 559 - protein, 21 aa, synthetic construct
  REGION 1..21: note = Description of Artificial Sequence: Synthetic peptide
FENRKGLSSHTRSHLRQMGVT

SEQ ID NO: 560 - protein, 21 aa, synthetic construct
  REGION 1..21: note = Description of Artificial Sequence: Synthetic peptide
APLEWLRYFDKKELELMLCGM

SEQ ID NO: 561 - protein, 21 aa, synthetic construct
  REGION 1..21: note = Description of Artificial Sequence: Synthetic peptide
LGITKTSKESTFKAARKYCPH

SEQ ID NO: 562 - protein, 21 aa, synthetic construct
  REGION 1..21: note = Description of Artificial Sequence: Synthetic peptide
YKNMRETLVYFTHLDYVDTEI

SEQ ID NO: 563 - protein, 21 aa, synthetic construct
  REGION 1..21: note = Description of Artificial Sequence: Synthetic peptide
ETSRNAGPSPVAQAPADRPVS

SEQ ID NO: 564 - protein, 21 aa, synthetic construct
  REGION 1..21: note = Description of Artificial Sequence: Synthetic peptide
VKQKGTGKGKDRTNTISMTGG

SEQ ID NO: 565 - protein, 21 aa, synthetic construct
  REGION 1..21: note = Description of Artificial Sequence: Synthetic peptide
QRIYHGKKPYKSSKSDKCFTH

SEQ ID NO: 566 - protein, 21 aa, synthetic construct
  REGION 1..21: note = Description of Artificial Sequence: Synthetic peptide
KIIGDASTQTNALKLPPSQPP

SEQ ID NO: 567 - DNA, 43 bp, synthetic construct
  misc_feature 1..43: note = Description of Artificial Sequence: Synthetic probe
  source 1..43: mol_type = other DNA
attattattattcaaatggatttatttatttatttatttattt

SEQ ID NO: 568 - DNA, 43 bp, synthetic construct
  misc_feature 1..43: note = Description of Artificial Sequence: Synthetic probe
  source 1..43: mol_type = other DNA
attattattatttaaatggatttatttatttatttatttattt

SEQ ID NO: 569 - DNA, 20 bp, synthetic construct
  misc_feature 1..20: note = Description of Artificial Sequence: Synthetic primer
  source 1..20: mol_type = other DNA
aagtgaaaatcaagcgcggg

SEQ ID NO: 570 - DNA, 20 bp, synthetic construct
  misc_feature 1..20: note = Description of Artificial Sequence: Synthetic primer
  source 1..20: mol_type = other DNA
caatttggcgacacagtcgg

SEQ ID NO: 571 - DNA, 1176 bp, Homo sapiens
  source 1..1176: mol_type = other DNA
atgaaccctcaaattcgcaatccgatggaacggatgtacagggacacattttacgacaattttgagaacgagcccatactctacggtaggagctatacgtggctttgttatgaagtgaaaatcaagcgcgggcgcagtaatctcctgtgggacaccggagtatttcgagggcaggtctatttcaaaccgcaataccatgctgagatgtgctttctgtcctggttctgtggaaatcagctgcccgcgtacaaatgctttcagataacatggttcgtctcctggaccccatgccccgactgtgtcgccaaattggctgaatttctttctgaacatccgaacgtgacgctcacaatcagcgcagctcggctgtattactactgggagcgggattacaggcgggctctttgtagattgtctcaggccggagctagggtcaagatcatggactatgaggagttcgcatactgttgggagaactttgtgtataacgaagggcagcagtttatgccgtggtataagtttgacgagaactatgccttcctgcatcggactttgaaagagatacttcgatatttgatggatcctgacacctttacttttaatttcaataatgacccccttgtcctgcggcgcagacagacatatctgtgctatgaagtagagcgccttgacaatgggacgtgggtgctgatggaccagcacatgggtttcctttgcaatgaagcaaaaaacctgctttgcggtttctacggtagacatgcggaactgcggttcttggatctcgtgcccagtctccagctggatcccgcgcaaatctatagggtaacttggttcatcagctggagtccatgtttctcatggggctgtgccggagaggtcagggcttttctccaagagaatactcatgttaggctccgcattttcgccgccagaatctatgactatgaccctctctataaagaagcgctccaaatgcttcgagacgccggcgcccaggtctccattatgacctacgacgaattcgagtattgctgggacacctttgtttataggcagggctgcccctttcagccatgggatgggctggaggagcactcacaagcactgagcggcagacttagagctatacttcaaaatcagggtaactacccatacgatgttccagattacgcttga

SEQ ID NO: 572 - DNA, 1176 bp, synthetic construct
  misc_feature 1..1176: note = Description of Artificial Sequence: Synthetic polynucleotide
  source 1..1176: mol_type = other DNA
atgaaccctcaaattcgcaatccgatggaacggatgtacagggacacattttacgacaattttgagaacgagcccatactctacggtaggagctatacgtggctttgttatgaagtgaaaatcaagcgcgggcgcagtaatctcctgtgggacaccggagtatttcgagggcaggtctatttcaaaccgcaataccatgctgcgatgtgctttctgtcctggttctgtggaaatcagctgcccgcgtacaaatgctttcagataacatggttcgtctcctggaccccatgccccgactgtgtcgccaaattggctgaatttctttctgaacatccgaacgtgacgctcacaatcagcgcagctcggctgtattactactgggagcgggattacaggcgggctctttgtagattgtctcaggccggagctagggtcaagatcatggactatgaggagttcgcatactgttgggagaactttgtgtataacgaagggcagcagtttatgccgtggtataagtttgacgagaactatgccttcctgcatcggactttgaaagagatacttcgatatttgatggatcctgacacctttacttttaatttcaataatgacccccttgtcctgcggcgcagacagacatatctgtgctatgaagtagagcgccttgacaatgggacgtgggtgctgatggaccagcacatgggtttcctttgcaatgaagcaaaaaacctgctttgcggtttctacggtagacatgcggcgctgcggttcttggatctcgtgcccagtctccagctggatcccgcgcaaatctatagggtaacttggttcatcagctggagtccatgtttctcatggggctgtgccggagaggtcagggcttttctccaagagaatactcatgttaggctccgcattttcgccgccagaatctatgactatgaccctctctataaagaagcgctccaaatgcttcgagacgccggcgcccaggtctccattatgacctacgacgaattcgagtattgctgggacacctttgtttataggcagggctgcccctttcagccatgggatgggctggaggagcactcacaagcactgagcggcagacttagagctatacttcaaaatcagggtaactacccatacgatgttccagattacgcttga

SEQ ID NO: 573 - protein, 21 aa, Homo sapiens
KFMWSEISYLAKWWDIIDIPK

SEQ ID NO: 574 - protein, 21 aa, synthetic construct
  REGION 1..21: note = Description of Artificial Sequence: Synthetic peptide
WMKNSLKVHSNSVLEQVWDIF

SEQ ID NO: 575 - protein, 21 aa, synthetic construct
  REGION 1..21: note = Description of Artificial Sequence: Synthetic peptide
TKEEENEMYNLTFFYENLKIP